European Patent Application EP 4 563 591 A1, published June 4, 2025. Title: Recombinant fusion protein for antigen delivery and uses thereof. Applicant: LG CHEM, LTD. The sequence listing filed with the application follows.

SEQUENCE LISTING (159 sequences)

SEQ ID NO: 1 - protein, 17 aa, Mus musculus
RNNSYTSYIMAICGMPL

SEQ ID NO: 2 - protein, 17 aa, Mus musculus
CWKYLSVQSQLFRGSSL

SEQ ID NO: 3 - protein, 17 aa, Mus musculus
GGISVKEHIEVNVVPLT

SEQ ID NO: 4 - protein, 17 aa, Mus musculus
MANQVIRCTAAVAWEAG

SEQ ID NO: 5 - protein, 17 aa, Mus musculus
PLEAMYMQWPVIAVNNG

SEQ ID NO: 6 - protein, 17 aa, Mus musculus
LHLEETLAGFWARLLER

SEQ ID NO: 7 - protein, 17 aa, Mus musculus
GGISVKEHIEVNVVPLT

SEQ ID NO: 8 - protein, 17 aa, Mus musculus
IYLESVAIMPQLFMVSK

SEQ ID NO: 9 - protein, 17 aa, Mus musculus
PLEAMYMQWPVIAVNNG

SEQ ID NO: 10 - protein, 23 aa, Mus musculus
TSTVQLIMQLMPFGCLLDYVREH

SEQ ID NO: 11 - protein, 15 aa, Mus musculus
QLIMQLMPFGCLLDY

SEQ ID NO: 12 - protein, 19 aa, Mus musculus
TVQLIMQLMPFGCLLDYVR

SEQ ID NO: 13 - protein, 11 aa, Mus musculus
IMQLMPFGCLL

SEQ ID NO: 14 - protein, 27 aa, Mus musculus
TPPPEEAMPFEFNGPAQGDHSQPPLQV

SEQ ID NO: 15 - protein, 27 aa, Mus musculus
FRRKAFLHWYTGEAMDEMEFTEAESNM

SEQ ID NO: 16 - protein, 27 aa, Mus musculus
SSPDEVALVEGVQSLGFTYLRLKDNYM

SEQ ID NO: 17 - protein, 27 aa, Mus musculus
PKPDFSQLQRNILPSNPRVTRFHINWD

SEQ ID NO: 18 - protein, 27 aa, Mus musculus
PSKPSFQEFVDWENVSPELNSTDQPFL

SEQ ID NO: 19 - protein, 15 aa, Mus musculus
DWENVSPELNSTDQP

SEQ ID NO: 20 - protein, 19 aa, Mus musculus
FVDWENVSPELNSTDQPFL

SEQ ID NO: 21 - protein, 23 aa, Mus musculus
QEFVDWENVSPELNSTDQPFLPS

SEQ ID NO: 22 - protein, 27 aa, Mus musculus
SFQEFVDWENVSPELNSTDQPFLPSAP

SEQ ID NO: 23 - protein, 27 aa, Mus musculus
EFKHIKAFDRTFANNPGPMVVFATPGM

SEQ ID NO: 24 - protein, 19 aa, Mus musculus
HGHSYTTAEELAGIGILTV

SEQ ID NO: 25 - protein, 27 aa, Mus musculus
YPKKGHGHSYTTAEELAGIGILTVILG

SEQ ID NO: 26 - protein, 23 aa, Mus musculus
HGHSYTTAEELAGIGILTVILGV

SEQ ID NO: 27 - protein, 27 aa, Mus musculus
DEVSGLEQLESIINFEKLTEWTSSNVM

SEQ ID NO: 28 - protein, 27 aa, Mus musculus
DKVSGLEQLESIINFEKLTEWTSSNVM

SEQ ID NO: 29 - protein, 27 aa, Mus musculus
DRVSGLEQLESIINFEKLTEWTSSNVM

SEQ ID NO: 30 - protein, 27 aa, Mus musculus
DRVKGLEQLESIINFEKLTEWTSSNVM

SEQ ID NO: 31 - protein, 8 aa, Mus musculus
SIINFEKL

SEQ ID NO: 32 - protein, 12 aa, Mus musculus
LESIINFEKLTE

SEQ ID NO: 33 - protein, 16 aa, Mus musculus
EQLESIINFEKLTEWT

SEQ ID NO: 34 - protein, 20 aa, Mus musculus
GLEQLESIINFEKLTEWTSS

SEQ ID NO: 35 - protein, 21 aa, Mus musculus
LCAGALVLAGGFFLLGFLFGW

SEQ ID NO: 36 - protein, 21 aa, Mus musculus
LSAGALVLAGGFFLLGFLFGW

SEQ ID NO: 37 - protein, 13 aa, Mus musculus
ALVLAGGFFLLGF

SEQ ID NO: 38 - protein, 17 aa, Mus musculus
AGALVLAGGFFLLGFLF

SEQ ID NO: 39 - protein, 9 aa, Mus musculus
VLAGGFFLL

SEQ ID NO: 40 - protein, 27 aa, Mus musculus
KKQFEELMLGEFLKLDRERAKNKIAKE

SEQ ID NO: 41 - protein, 27 aa, Mus musculus
GSNGDPSSPYSLHYLSPTGVNEYLTAL

SEQ ID NO: 42 - protein, 27 aa, Mus musculus
PGDSQNAAKARDETAALLNSAVLGAAP

SEQ ID NO: 43 - protein, 27 aa, Mus musculus
HVLSKLLSFMAPIDHTTMSDDARTELF

SEQ ID NO: 44 - protein, 27 aa, Mus musculus
EAYEEDRETFMNKFIYEIARRHPFLYA

SEQ ID NO: 45 - protein, 98 aa, synthetic construct
MIPGGLSEAKPATPEIQEIVDKVKPQLEEKTNETYGKLEAVQYKTQVVAGTNYYIKVRAGDNKYMHLKVFKSLPGQNEDLVLTGYQVDKNKDDELTGF

SEQ ID NO: 46 - protein, 99 aa, synthetic construct
MIPGGLSEAKPATPEIQEIVDKVKPQLEEKTNETYGKLEAVQYKTQVVAGTNYYIKVRAGDNKYMHLKVFKSLPGQNEDLVLTGYSQVDKNKDDELTGF

SEQ ID NO: 47 - protein, 105 aa, synthetic construct
MVKQIESKTAFQEALDAAGDKLVVVDFSATWCGPCKMIKPFFHSLSEKYSNVIFLEVDVDDSQDVASESEVKSMPTFQFFKKGQKVGEFSGANKEKLEATINELV

SEQ ID NO: 48 - protein, 105 aa, synthetic construct
MVKQIESKTAFQEALDAAGDKLVVVDFSATWCGPCKMIKPFFHSLSEKYSNVIFLEVDVDDCQDVASECEVKSMPTFQFFKKGQKVGEFSGANKEKLEATINELV

SEQ ID NO: 49 - protein, 105 aa, synthetic construct
MVKQIESKTAFQEALDAAGDKLVVVDFSATWSGPSKMIKPFFHSLSEKYSNVIFLEVDVDDSQDVASESEVKSMPTFQFFKKGQKVGEFSGANKEKLEATINELV

SEQ ID NO: 50 - protein, 105 aa, synthetic construct
MVKQIESKTAFQEALDAAGDKLVVVDFSATWCGPCKMIKPFFHSLSEKYSNVIFLEVDVDDCQDVASECEVKCMPTFQFFKKGQKVGEFSGANKEKLEATINELV

SEQ ID NO: 51 - protein, 99 aa, synthetic construct
MIPGGLTEARPATAEVQEIADRVKAQLEEETNEKYEIFKAVQYKTQVGGGGGVNYFIKMDVGGGCFTHIKVFKDLSGKNNLELTGYQTNKTEDDELTYF

SEQ ID NO: 52 - protein, 97 aa, synthetic construct
MIPGGLTEARPATAEVQEIADRVKAQLEEETNEKYEIFKAVQYKTQVVAGVNYFIKMDVGGGCFTHIKVFKDLSGKNNLELTGYQTNKTEDDELTYF

SEQ ID NO: 53 - protein, 117 aa, synthetic construct
MAVYVKFKVPEEIQKELLDAVAKAQKIKKAANEVTKAVERGIAKLVIIAEDVKPEELVAHLPYLCEEKGIPYAYVASKQDLGKAAGLEVAASSVAIINEGDAEELKVLIEKVNVLKQ

SEQ ID NO: 54 - protein, 67 aa, synthetic construct
MKMIKVKVVGRNIEKEIEWREGMKVRDILRAVGFNTESAVAKVNGKVVLEDDEVKDGDFVEVIPVWT

SEQ ID NO: 55 - protein, 92 aa, synthetic construct
MPPKDLVVTEVTEETVNLAWDNEMRVTEYLVVYTPTHEGGLEMQFRVPGDQTSTIIQELEPGVEYFIRVFAILENKKSIPVSARVATYLPAP

SEQ ID NO: 56 - protein, 90 aa, synthetic construct
MEGLKFKSIKETSVEVEWDPLDIAFETWEIIFRNMNKEDEGEITKSLRRPETSYRQTGLAPGQEYEISLHIVKNNTRGPGLKRVTTTRLD

SEQ ID NO: 57 - protein, 187 aa, synthetic construct
MAPSQIEVKDVTDTTALITWFKPLAEIDGIELTYGIKDVPGDRTTIDLTEDENQYSIGNLKPDTEYEVSLISRRGDMSSNPAKETFTTGLDAPRNLRRVSQTDNSITLEWRNGKAAIDSYRIKYAPISGGDHAEVDVPKSQQATTKTTLTGLRPGTEYGIGVSAVKEDKESNPATINAATELDTPKD

SEQ ID NO: 58 - protein, 91 aa, synthetic construct
MAPSQIEVKDVTDTTALITWFKPLAEIDGIELTYGIKDVPGDRTTIDLTEDENQYSIGNLKPDTEYEVSLISRRGDMSSNPAKETFTTGLD

SEQ ID NO: 59 - protein, 189 aa, synthetic construct
MLDAPSQIEVKDVTDTTALITWFKPLAEIDGIELTYGIKDVPGDRTTIDLTEDENQYSIGNLKPDTEYEVSLISRRGDMSSNPAKETFTTGLDAPRNLRRVSQTDNSITLEWRNGKAAIDSYRIKYAPISGGDHAEVDVPKSQQATTKTTLTGLRPGTEYGIGVSAVKEDKESNPATINAATELDTPKD

SEQ ID NO: 60 - protein, 92 aa, synthetic construct
MLDAPSQIEVKDVTDTTALITWFKPLAEIDGIELTYGIKDVPGDRTTIDLTEDENQYSIGNLKPDTEYEVSLISRRGDMSSNPAKETFTTGL

SEQ ID NO: 61 - protein, 97 aa, synthetic construct
MAPRNLRRVSQTDNSITLEWRNGKAAIDSYRIKYAPISGGDHAEVDVPKSQQATTKTTLTGLRPGTEYGIGVSAVKEDKESNPATINAATELDTPKD

SEQ ID NO: 62 - protein, 89 aa, synthetic construct
MEVKIEKPTPEKLKELSVEKWPIWEKEVSEFDWYYDTNRTAYILEGKVEVTTEDGKKYVIEKGDLVTFPKGLRSRWKVLEPVRMHYNLF

SEQ ID NO: 63 - protein, 109 aa, synthetic construct
MSDKIIHLTDDSFDTDVLKADGAILVDFWAEWSGPSKMIAPILDEIADEYQGKLTVAKLNIDQNPGTAPKYGIRGIPTLLLFKNGEVAATKVGALSKGQLKEFLDANLA

SEQ ID NO: 64 - protein, 109 aa, synthetic construct
MSDKIIHLTDDSFDTDVLKADGAILVDFWAEWCGPCKMIAPILDEIADEYQGKLTVAKLNIDQNPGTAPKYGIRGIPTLLLFKNGEVAATKVGALSKGQLKEFLDANLA

SEQ ID NO: 65 - protein, 90 aa, synthetic construct
MKIEYFKNDKSSVSKAMLPKIQTIAKNFDIDIEVIDVIENPSYPAQKLVFTVPTVIILDKEFEIKRFARNFSISEVINTIERYLEISNKE

SEQ ID NO: 66 - protein, 40 aa, synthetic construct
VIAMPSVRKYAREKGVDIRLVQGTGKNGRVLKEDIDAWLA

SEQ ID NO: 67 - protein, 40 aa, synthetic construct
VIAMPSVRKYAREKGVDIRLVQGTGKGGRVLKEDIDAWLA

SEQ ID NO: 68 - protein, 152 aa, synthetic construct
MANLERTFIAIKPDGVQRGLVGEIIKRFEQKGFRLVAMKFLRASEEHLKQHYIDLKDRPFFPGLVKYMNSGPVVAMVWEGLNVVKTGRVMLGETNPADSKPGTIRGDFCIQVGRNIIHGSDSVESAEKEIHLWFKPEELIDYKSCAHDWVYE

SEQ ID NO: 69 - protein, 15 aa, synthetic construct
QYIKANSKFIGITEL

SEQ ID NO: 70 - protein, 5 aa, synthetic construct
GGGGS

SEQ ID NO: 71 - protein, 4 aa, synthetic construct
SSGG

SEQ ID NO: 72 - protein, 5 aa, synthetic construct
GGGGG

SEQ ID NO: 73 - protein, 10 aa, synthetic construct
GGGGSGGGGG

SEQ ID NO: 74 - DNA, 291 bp, synthetic construct
  source 1..291: mol_type = other DNA
atgatcccaggtggtctgaccgaagcgcgcccggcgaccgcggaagtgcaggaaattgcggatcgcgtgaaagcgcagctggaagaagaaaccaacgaaaaatatgaaatttttaaagccgttcagtacaaaacccaggtcgtagcgggtgtgaactattttattaaaatggatgtgggcggcggctgctttacccatattaaagtgtttaaagatctgagcggcaaaaacaacctggaactgaccggctatcagaccaacaaaaccgaagatgatgaactgacctatttt

SEQ ID NO: 75 - DNA, 294 bp, synthetic construct
  source 1..294: mol_type = other DNA
atgatcccaggaggtctgtctgaagctaagcctgcaacgccggaaattcaagaaattgttgacaaagtgaagccgcagctggaagagaaaaccaacgaaacctacggtaagctggaagccgttcagtacaaaacccaggtcgtagcgggtaccaattactatatcaaagtgcgtgcgggtgacaacaagtatatgcacctgaaagttttcaaaagcctcccgggacagaatgaagatctggtcttgactggttatcaagtggacaagaacaaagatgatgagctgacgggtttt

SEQ ID NO: 76 - DNA, 315 bp, synthetic construct
  source 1..315: mol_type = other DNA
atggttaaacaaattgagtcgaaaaccgccttccaagaagctcttgatgctgctggtgataagttggtcgtagttgacttctcagccacttggtgcggtccatgcaaaatgataaagccttttttccactcgttgagtgagaagtattcaaacgtaatttttttagaagtggatgtcgatgattcacaagatgttgcaagtgagagcgaagtcaagtctatgcccacgtttcaatttttcaaaaaaggtcagaaggtgggcgagttttcaggtgctaataaagaaaaattagaagctacgattaatgaactggtc

SEQ ID NO: 77 - DNA, 315 bp, synthetic construct
  source 1..315: mol_type = other DNA
atggttaaacaaattgagtcgaaaaccgccttccaagaagctcttgatgctgctggtgataagttggtcgtagttgacttctcagccacttggtgcggtccatgcaaaatgataaagccttttttccactcgttgagtgagaagtattcaaacgtaatttttttagaagtggatgtcgatgattgccaagatgttgcaagtgagtgcgaagtcaagtctatgcccacgtttcaatttttcaaaaaaggtcagaaggtgggcgagttttcaggtgctaataaagaaaaattagaagctacgattaatgaactggtc

SEQ ID NO: 78 - DNA, 315 bp, synthetic construct
  source 1..315: mol_type = other DNA
atggttaaacaaattgagtcgaaaaccgccttccaagaagctcttgatgctgctggtgataagttggtcgtagttgacttctcagccacttggtctggtccatctaaaatgataaagccttttttccactcgttgagtgagaagtattcaaacgtaatttttttagaagtggatgtcgatgattcacaagatgttgcaagtgagagcgaagtcaagtctatgcccacgtttcaatttttcaaaaaaggtcagaaggtgggcgagttttcaggtgctaataaagaaaaattagaagctacgattaatgaactggtc

SEQ ID NO: 79 - DNA, 297 bp, synthetic construct
  source 1..297: mol_type = other DNA
atgatcccaggtggtctgaccgaagcgcgcccggcgaccgcggaagtgcaggaaattgcggatcgcgtgaaagcgcagctggaagaagaaaccaacgaaaaatatgaaatttttaaagccgttcagtacaaaacccaggtcggcggcggcgggggggtgaactattttattaaaatggatgtgggcggcggctgctttacccatattaaagtgtttaaagatctgagcggcaaaaacaacctggaactgaccggctatcagaccaacaaaaccgaagatgatgaactgacctatttt

SEQ ID NO: 80 - DNA, 201 bp, synthetic construct
  source 1..201: mol_type = other DNA
atgaagatgatcaaggttaaagtagttggtcgtaacatcgagaaagagatcgaatggcgcgagggtatgaaagtgcgtgacattctgcgtgcagttggtttcaacaccgagtctgctgtagcaaaagtgaacggtaaagtcgtgctggaagacgacgaagtaaaagatggtgacttcgtggaagttattccggtttggact

SEQ ID NO: 81 - DNA, 273 bp, synthetic construct
  source 1..273: mol_type = other DNA
ccaccgaaagacctggttgttaccgaggtgactgaggaaaccgttaatctggcctgggacaacgaaatgcgtgtcaccgagtatctggttgtgtatactccgacccatgaaggtggcctggaaatgcagttccgtgttccgggcgatcagaccagcaccatcatccaggaactggagccaggcgtggagtatttcatccgtgttttcgccatcctggaaaataaaaaatctatcccggtttccgcgcgtgtagcgacctatctgccagcaccg

SEQ ID NO: 82 - DNA, 267 bp, synthetic construct
  source 1..267: mol_type = other DNA
gaaggcctgaaattcaaaagcatcaaagagacctccgttgaagtagaatgggacccgctggacatcgcttttgaaacctgggaaatcattttccgcaacatgaacaaagaggatgaaggtgaaatcacgaaaagcctgcgtcgtccggaaacctcttatcgtcagactggtctggctccgggccaggaatatgaaatctctctgcacatcgtgaaaaacaacactcgcggtcctggtctgaaacgtgtcactactactcgtctggac

SEQ ID NO: 83 - DNA, 558 bp, synthetic construct
  source 1..558: mol_type = other DNA
gctccgtcccagatcgaagtgaaggacgtaacggataccaccgcactgatcacttggttcaaaccgctggcagaaattgatggcattgaactgacctatggcatcaaagacgtgccgggtgaccgtaccaccattgatctgacggaagatgagaaccagtattccatcggcaacctgaaaccggacacggaatacgaagtgtctctgatctcccgtcgcggcgacatgtcctctaacccggctaaagaaactttcactaccggtctggatgcaccgcgcaacctgcgtcgtgtatctcagaccgataactctattaccctggaatggcgtaatggtaaagctgcgatcgactcctaccgtatcaaatacgcgccgatctccggtggtgatcatgcagaagtagatgtacctaaatctcagcaggctacgacgaaaaccactctgactggcctgcgtccgggtactgagtatggtatcggtgtttctgctgttaaagaagataaagaatccaacccagcgaccatcaacgcggctactgaactggatacgccaaaagat

SEQ ID NO: 84 - DNA, 270 bp, synthetic construct
  source 1..270: mol_type = other DNA
gctccgtcccagatcgaagtgaaggacgtaacggataccaccgcactgatcacttggttcaaaccgctggcagaaattgatggcattgaactgacctatggcatcaaagacgtgccgggtgaccgtaccaccattgatctgacggaagatgagaaccagtattccatcggcaacctgaaaccggacacggaatacgaagtgtctctgatctcccgtcgcggcgacatgtcctctaacccggctaaagaaactttcactaccggtctggat

SEQ ID NO: 85 - DNA, 564 bp, synthetic construct
  source 1..564: mol_type = other DNA
ctggatgctccgtcccagatcgaagtgaaggacgtaacggataccaccgcactgatcacttggttcaaaccgctggcagaaattgatggcattgaactgacctatggcatcaaagacgtgccgggtgaccgtaccaccattgatctgacggaagatgagaaccagtattccatcggcaacctgaaaccggacacggaatacgaagtgtctctgatctcccgtcgcggcgacatgtcctctaacccggctaaagaaactttcactaccggtctggatgcaccgcgcaacctgcgtcgtgtatctcagaccgataactctattaccctggaatggcgtaatggtaaagctgcgatcgactcctaccgtatcaaatacgcgccgatctccggtggtgatcatgcagaagtagatgtacctaaatctcagcaggctacgacgaaaaccactctgactggcctgcgtccgggtactgagtatggtatcggtgtttctgctgttaaagaagataaagaatccaacccagcgaccatcaacgcggctactgaactggatacgccaaaagat

SEQ ID NO: 86 - DNA, 273 bp, synthetic construct
  source 1..273: mol_type = other DNA
ctggatgctccgtcccagatcgaagtgaaggacgtaacggataccaccgcactgatcacttggttcaaaccgctggcagaaattgatggcattgaactgacctatggcatcaaagacgtgccgggtgaccgtaccaccattgatctgacggaagatgagaaccagtattccatcggcaacctgaaaccggacacggaatacgaagtgtctctgatctcccgtcgcggcgacatgtcctctaacccggctaaagaaactttcactaccggtctg

SEQ ID NO: 87 - DNA, 288 bp, synthetic construct
  source 1..288: mol_type = other DNA
gcaccgcgcaacctgcgtcgtgtatctcagaccgataactctattaccctggaatggcgtaatggtaaagctgcgatcgactcctaccgtatcaaatacgcgccgatctccggtggtgatcatgcagaagtagatgtacctaaatctcagcaggctacgacgaaaaccactctgactggcctgcgtccgggtactgagtatggtatcggtgtttctgctgttaaagaagataaagaatccaacccagcgaccatcaacgcggctactgaactggatacgccaaaagat

SEQ ID NO: 88 - DNA, 267 bp, synthetic construct
  source 1..267: mol_type = other DNA
atggaagttaaaatcgagaaaccgactccggaaaaactgaaggaactgtctgtcgaaaagtggccgatctgggagaaagaagtgtctgagttcgactggtactacgataccaaccgtactgcatacatcctggagggcaaggttgaagttaccaccgaagatggtaagaaatacgttatcgaaaaaggcgacctggtaacttttcctaaaggcctgcgttctcgttggaaagttctggaacctgttcgtatgcactacaacctgttc

SEQ ID NO: 89 - DNA, 327 bp, synthetic construct
  source 1..327: mol_type = other DNA
atgagcgataaaattattcacctgactgacgacagttttgacacggatgtactcaaagcggacggggcgatcctcgtcgatttctgggcagagtggtctggtccgtctaaaatgatcgccccgattctggatgaaatcgctgacgaatatcagggcaaactgaccgttgcaaaactgaacatcgatcaaaaccctggcactgcgccgaaatatggcatccgtggtatcccgactctgctgctgttcaaaaacggtgaagtggcggcaaccaaagtgggtgcactgtctaaaggtcagttgaaagagttcctcgacgctaacctggcc

SEQ ID NO: 90 - protein, 109 aa, synthetic construct; identical to SEQ ID NO: 64

SEQ ID NO: 91 - DNA, 270 bp, synthetic construct
  source 1..270: mol_type = other DNA
atgaaaatcgaatactttaagaatgacaaaagctctgttagcaaagctatgctgccgaaaatccaaactattgcaaaaaactttgatattgatattgaggtaattgacgttatagaaaatccttcttatccagctcaaaaactggtttttacagtaccaacagtaatcattctggataaagaatttgaaatcaaacgttttgcacgtaattttagtattagtgaagtaatcaatacaattgaacgttacctggaaataagtaataaagaa

SEQ ID NO: 92 - protein, 40 aa, synthetic construct; identical to SEQ ID NO: 66

SEQ ID NO: 93 - protein, 40 aa, synthetic construct; identical to SEQ ID NO: 67

SEQ ID NO: 94 - DNA, 65 bp, synthetic construct
  source 1..65: mol_type = other DNA
gcgtctagaaataattttgtttaactttaagaaggagatatacatatggcagatctcaattggat

SEQ ID NO: 95 - DNA, 25 bp, synthetic construct
  source 1..25: mol_type = other DNA
cagcggtttctttaccagactcgag

SEQ ID NO: 96 - DNA, 33 bp, synthetic construct
  source 1..33: mol_type = other DNA
gcgcatatgcagatttttgtgaaaaccctgacc

SEQ ID NO: 97 - DNA, 27 bp, synthetic construct
  source 1..27: mol_type = other DNA
gactagttctagagtcgacgagctctc

SEQ ID NO: 98 - DNA, 43 bp, synthetic construct
  source 1..43: mol_type = other DNA
tagcgcatatggaagttaaaatcgagaaaccgactccggaaaa

SEQ ID NO: 99 - DNA, 49 bp, synthetic construct
  source 1..49: mol_type = other DNA
agagacccgcaacgctgggtctcagaacaggttgtagtgcatacgaaca

SEQ ID NO: 100 - DNA, 48 bp, synthetic construct
  source 1..48: mol_type = other DNA
agagacccgcaacgctgggtctcaggtggtggtggaggagttatcgct

SEQ ID NO: 101 - DNA, 74 bp, synthetic construct
  source 1..74: mol_type = other DNA
cgacgagctctcaatggtggtgatggtgatgtccgccagccagccacgcgtcgatgtcttctttcagaacacgg

SEQ ID NO: 102 - DNA, 85 bp, synthetic construct
  source 1..85: mol_type = other DNA
aggaccgagcaaaccgtcgtttcaggaatttgtggactgggaaaacgtgtcgccggaactgaacagcaccgatcagccgtttctg

SEQ ID NO: 103 - DNA, 85 bp, synthetic construct
  source 1..85: mol_type = other DNA
cacccagaaacggctgatcggtgctgttcagttccggcgacacgttttcccagtccacaaattcctgaaacgacggtttgctcgg

SEQ ID NO: 104 - DNA, 74 bp, synthetic construct
  source 1..74: mol_type = other DNA
gctcaccataaacagctgcggcataatcgccacgctttccagataaattcctccaccaccaccgaacaggttgt

SEQ ID NO: 105 - DNA, 88 bp, synthetic construct
  source 1..88: mol_type = other DNA
gcgattatgccgcagctgtttatggtgagcaaaggcggtggtggaggagttatcgctatgccgtccgtacgcaaatatgcacgtgaaa

SEQ ID NO: 106 - DNA, 63 bp, synthetic construct
  source 1..63: mol_type = other DNA
tttaccggtaccctgaaccaggcggatatcaacgcctttttcacgtgcatatttgcgtacgga

SEQ ID NO: 107 - DNA, 88 bp, synthetic construct
  source 1..88: mol_type = other DNA
gcaaatatgcacgtgaaaaaggcgttgatatccgcctggttcagggtaccggtaaaaacggccgtgttctgaaagaagacatcgacgc

SEQ ID NO: 108 - DNA, 32 bp, synthetic construct
  source 1..32: mol_type = other DNA
gcgcatatggttaaacaaattgagtcgaaaac

SEQ ID NO: 109 - DNA, 48 bp, synthetic construct
  source 1..48: mol_type = other DNA
tatcattttagatggaccagaccaagtggctgagaagtcaactacgac

SEQ ID NO: 110 - DNA, 51 bp, synthetic construct
  source 1..51: mol_type = other DNA
cacttggtctggtccatctaaaatgataaagccttttttccactcgttgag

SEQ ID NO: 111 - DNA, 47 bp, synthetic construct
  source 1..47: mol_type = other DNA
tgagacccagcgttgcgggtctcttcctccaccaccaccgaccagtt

SEQ ID NO: 112 - DNA, 48 bp, synthetic construct; identical to SEQ ID NO: 100
  source 1..48: mol_type = other DNA

SEQ ID NO: 113 - DNA, 89 bp, synthetic construct
  source 1..89: mol_type = other DNA
ccggtaccctgaaccaggcggatatcaacgcctttttcacgtgcatatttgcgtacggacggcatagcgataactcctccaccaccacc

SEQ ID NO: 114 - DNA, 88 bp, synthetic construct; identical to SEQ ID NO: 107
  source 1..88: mol_type = other DNA

SEQ ID NO: 115 - DNA, 85 bp, synthetic construct
  source 1..85: mol_type = other DNA
aggaaccccgccgccggaagaagcgatgccgtttgaatttaatggtccggcgcagggtgatcatagccagccgccgctgcaggtg

SEQ ID NO: 116 - DNA, 85 bp, synthetic construct
  source 1..85: mol_type = other DNA
cacccacctgcagcggcggctggctatgatcaccctgcgccggaccattaaattcaaacggcatcgcttcttccggcggcggggt

SEQ ID NO: 117 - DNA, 55 bp, synthetic construct
  source 1..55: mol_type = other DNA
aggactgcatctggaagaaaccctggcgggcttttgggcgcgcctgctggaacgc

SEQ ID NO: 118 - DNA, 55 bp, synthetic construct
  source 1..55: mol_type = other DNA
caccgcgttccagcaggcgcgcccaaaagcccgccagggtttcttccagatgcag

SEQ ID NO: 119 - DNA, 69 bp, synthetic construct
  source 1..69: mol_type = other DNA
gcaaatttattggcattaccgaactgggcggcggcgggtctatggttaaacaaattgagtcgaaaaccg

SEQ ID NO: 120 - DNA, 30 bp, synthetic construct
  source 1..30: mol_type = other DNA
ttcgccaatccggatatagttcctcctttc

SEQ ID NO: 121 - DNA, 55 bp, synthetic construct
  source 1..55: mol_type = other DNA
gcggcatatgcagtatattaaagcgaacagcaaatttattggcattaccgaactg

SEQ ID NO: 122 - DNA, 55 bp, synthetic construct
  source 1..55: mol_type = other DNA
aggaatttatctggaaagcgtggcgattatgccgcagctgtttatggtgagcaaa

SEQ ID NO: 123 - DNA, 55 bp, synthetic construct
  source 1..55: mol_type = other DNA
cacctttgctcaccataaacagctgcggcataatcgccacgctttccagataaat

SEQ ID NO: 124 - DNA, 76 bp, synthetic construct
  source 1..76: mol_type = other DNA
gcgactagtaataattttgtttaactttaagaaggagatataccatgatcccaggaggtctgtctgaagctaagcc

SEQ ID NO: 125 - DNA, 63 bp, synthetic construct
  source 1..63: mol_type = other DNA
ctgttccagaccgctaacttcatcggatccaccaccaccaaaacccgtcagctcatcatcttt

SEQ ID NO: 126 - DNA, 33 bp, synthetic construct
  source 1..33: mol_type = other DNA
ggtggatccgatgaagttagcggtctggaacag

SEQ ID NO: 127 - DNA, 69 bp, synthetic construct
  source 1..69: mol_type = other DNA
gacgagctctcagtgatgatggtggtgatgacctccactagacataacattgctgctggtccattcggt

SEQ ID NO: 128 - DNA, 29 bp, synthetic construct
  source 1..29: mol_type = other DNA
gcgggatccagcagcccggatgaagtggc

SEQ ID NO: 129 - DNA, 73 bp, synthetic construct
  source 1..73: mol_type = other DNA
cgcgagctctcagtgatgatggtggtgatgacctcccatataattatctttcagacgcagataggtaaaaccc

SEQ ID NO: 130 - DNA, 49 bp, synthetic construct
  source 1..49: mol_type = other DNA
gcgcatatgggcggcggcgggtctatgatcccaggaggtctgtctgaag

SEQ ID NO: 131 - DNA, 25 bp, synthetic construct
  source 1..25: mol_type = other DNA
gtccggcgtagaggatcgagatctc

SEQ ID NO: 132 - DNA, 70 bp, synthetic construct
  source 1..70: mol_type = other DNA
gcgtacggacggcatagcgataactcctccaccaccacccatataattatctttcagacgcagataggta

SEQ ID NO: 133 - DNA, 26 bp, synthetic construct
  source 1..26: mol_type = other DNA
ggtggtggtggaggagttatcgctat

SEQ ID NO: 134 - DNA, 88 bp, synthetic construct
  source 1..88: mol_type = other DNA
gatccatttatctggaaagcgtggcgattatgccgcagctgtttatggtgagcaaaggcggacatcaccatcaccaccattgagagct

SEQ ID NO: 135 - DNA, 80 bp, synthetic construct
  source 1..80: mol_type = other DNA
ctcaatggtggtgatggtgatgtccgcctttgctcaccataaacagctgcggcataatcgccacgctttccagataaatg

SEQ ID NO: 136 - DNA, 63 bp, synthetic construct
  source 1..63: mol_type = other DNA
gcgtacggacggcatagcgataactcctccaccaccacctttgctcaccataaacagctgcgg

SEQ ID NO: 137 - DNA, 85 bp, synthetic construct
  source 1..85: mol_type = other DNA
aggagaatttaaacatattaaagcgtttgatcgtacctttgcgaataacccgggtccgatggtggtgtttgcgaccccgggtatg

SEQ ID NO: 138 - DNA, 85 bp, synthetic construct
  source 1..85: mol_type = other DNA
cacccatacccggggtcgcaaacaccaccatcggacccgggttattcgcaaaggtacgatcaaacgctttaatatgtttaaattc

SEQ ID NO: 139 - DNA, 70 bp, synthetic construct
  source 1..70: mol_type = other DNA
gcaaatttattggcattaccgaactgggcggcggcgggtctatggaagttaaaatcgagaaaccgactcc

SEQ ID NO: 140 - DNA, 55 bp, synthetic construct; identical to SEQ ID NO: 117
  source 1..55: mol_type = other DNA

SEQ ID NO: 141 - DNA, 55 bp, synthetic construct; identical to SEQ ID NO: 118
  source 1..55: mol_type = other DNA

SEQ ID NO: 142 - DNA, 44 bp, synthetic construct
  source 1..44: mol_type = other DNA
tcagggtaccggtaaaggtggccgtgttctgaaagaagacatcg

SEQ ID NO: 143 - DNA, 82 bp, synthetic construct
  source 1..82: mol_type = other DNA
tgagacccagcgttgcgggtctctgccgccaccgccaccgcttccaccaccaccgaccagttcattaatcgtagcttctaat

SEQ ID NO: 144 - DNA, 82 bp, synthetic construct
  source 1..82: mol_type = other DNA
agagacccgcaacgctgggtctcaggcggtggcggtggtagcggtggtggaggagttatcgctatgccgtccgtacgcaaat

SEQ ID NO: 145 - DNA, 81 bp, synthetic construct
  source 1..81: mol_type = other DNA
tgagacccagcgttgcgggtctcttcctccaccaccaccgcttccaccaccaccgaacaggttgtagtgcatacgaacagg

SEQ ID NO: 146 - DNA, 82 bp, synthetic construct
  source 1..82: mol_type = other DNA
agagacccgcaacgctgggtctcaggtggcggcggtggtagcggtggtggaggagttatcgctatgccgtccgtacgcaaat

SEQ ID NO: 147 - DNA, 85 bp, synthetic construct
  source 1..85: mol_type = other DNA
aggaagcagcccggatgaagtggcgctggttgaaggtgtgcagagcctgggttttacctatctgcgtctgaaagataattatatg

SEQ ID NO: 148 - DNA, 85 bp, synthetic construct
  source 1..85: mol_type = other DNA
cacccatataattatctttcagacgcagataggtaaaacccaggctctgcacaccttcaaccagcgccacttcatccgggctgct

SEQ ID NO: 149 - DNA, 74 bp, synthetic construct
  source 1..74: mol_type = other DNA
gcgcatatgcagtatattaaagcgaacagcaaatttattggcattaccgaactgggcggcggcgggtctatgat

SEQ ID NO: 150 - DNA, 85 bp, synthetic construct
  source 1..85: mol_type = other DNA
cggccatgtgctgagcaaactgctgagctttatggcgccgattgatcataccaccatgagcgatgatgcgcgcaccgaactgttt

SEQ ID NO: 151 - DNA, 85 bp, synthetic construct
  source 1..85: mol_type = other DNA
caccaaacagttcggtgcgcgcatcatcgctcatggtggtatgatcaatcggcgccataaagctcagcagtttgctcagcacatg

SEQ ID NO: 152 - DNA, 85 bp, synthetic construct
  source 1..85: mol_type = other DNA
cggcggcagcaacggcgatccgagcagcccgtatagcctgcattatctgagcccgaccggcgtgaacgaatatctgaccgcgctg

SEQ ID NO: 153 - DNA, 85 bp, synthetic construct
  source 1..85: mol_type = other DNA
cacccagcgcggtcagatattcgttcacgccggtcgggctcagataatgcaggctatacgggctgctcggatcgccgttgctgcc

SEQ ID NO: 154 - DNA, 85 bp, synthetic construct
  source 1..85: mol_type = other DNA
cggcccgggcgatagccagaacgcggcgaaagcgcgcgatgaaaccgcggcgctgctgaacagcgcggtgctgggcgcggcgccg

SEQ ID NO: 155 - DNA, 85 bp, synthetic construct
  source 1..85: mol_type = other DNA
cacccggcgccgcgcccagcaccgcgctgttcagcagcgccgcggtttcatcgcgcgctttcgccgcgttctggctatcgcccgg

SEQ ID NO: 156 - DNA, 55 bp, synthetic construct
  source 1..55: mol_type = other DNA
aggaggcggcattagcgtgaaagaacatattgaagtgaacgtggtgccgctgacc

SEQ ID NO: 157 - DNA, 55 bp, synthetic construct
  source 1..55: mol_type = other DNA
caccggtcagcggcaccacgttcacttcaatatgttctttcacgctaatgccgcc

SEQ ID NO: 158 - DNA, 55 bp, synthetic construct
  source 1..55: mol_type = other DNA
aggaccgctggaagcgatgtatatgcagtggccggtgattgcggtgaacaacggc

SEQ ID NO: 159 - DNA, 55 bp, synthetic construct
  source 1..55: mol_type = other DNA
caccgccgttgttcaccgcaatcaccggccactgcatatacatcgcttccagcgg